European Patent Application EP 4 574 989 A1, published June 25, 2025. Title: ALPHA-L-FUCOSIDASES AND USES THEREOF. Applicant: Vilnius University. Application EP. The sequence listing filed with the application follows.

SEQUENCE LISTING (8 sequences)

SEQ ID NO: 1 - protein, 569 aa, unidentified
MDKMWGDSKSKATQSDLTRGPSLREGRYGMFIHWGLYSSLGGKWKDKTYYGIGEWIMNPAMAGIPVEDYMEPAKSFNPEQFDAKAIVQLAKDAGMKYIIITSKHHEGFAMFKSAHPFNIVDASPFQRDPMKELSDACRAAGLGFGFYYSHFQDWTSPGGHGGPSKNADGSDATFEKYFREKCYPQVKEICTQYGPLDVIWFDTPGSMPKELVVELHDLVRSTQPKALLGSRIGHGMGDYESLGDMEVPPERVDGFWESCDTTNDSWSYAWYDTNWKSPKVILHRLVSTVARGGNYLLNIGPDGKGAVPAECQEFLKQAGTWLKAHPEVISESGPSPWRYAMPWGDITVRKDGKLNLVVFDLPQDGFIYLPGLSTPVKSASLIDTGRKTLVKTELFGKSMRIKLPERCRTAIATLVELQLTSAPEVDQSVTVHPNTPNDLLVHFAEVMGAEKKKTNWMAKFGEWKHATQISRWTPGGKARWTANFLQPGFYQVTAKYRGEMDPKSRVTWRITTNEANSIQNQQPVTGQYQSMPMGVFEVKMPGKRVIEVSLVDGDLDATSLESIGMTLIR

SEQ ID NO: 2 - protein, 430 aa, unidentified
MQKDFLNETTQDRDARMQWWRDATFGMFIHWGAYAVPAGEYKGKVVNGVGEWIMHTANIPIPEYEEYVRQFNPLQFDAKEWVRIAKDAGMKYIVITSKHHDGFSLWDSKVSNYDVMDASPFKRDILKELSDACKEAGIKMCFYHSIMDWHEPDAESKKEYTHQNAPNPDFARYREQFLKPQLKELVEKYDPAVLWFDGEWIPEWTEEQGRDLYNYLRNLKPDLVINNRVGKGRAGMQGMNLYKNAAGDFGTPEQEILEGTSDTDWESCMTMNDSWGFKKTDHNWKSAELLIHNLVDIAAKGGNYLLNVGPTAQGLIPVASVDRLREMGEWMKINNEAIYATNSTKKYKEGEVKYTVSKDGNFVYAIVTKAVSGELVLHNVDLKRGSNIYMLGANKPLKYKADASGSLHIEWPKDLPCKYAWTLKITGSPK

SEQ ID NO: 3 - DNA, 20 bp, synthetic construct
  source 1..20: mol_type = other DNA
taatacgactcactataggg

SEQ ID NO: 4 - DNA, 24 bp, synthetic construct
  source 1..24: mol_type = other DNA
gagcggataacaatttcacacagg

SEQ ID NO: 5 - DNA, 42 bp, synthetic construct
  source 1..42: mol_type = other DNA
agaaggagatataactatggacaagatgtggggggactcgaa

SEQ ID NO: 6 - DNA, 43 bp, synthetic construct
  source 1..43: mol_type = other DNA
gtggtggtgatggtgatggccgcgaatgagtgtcatgcctatg

SEQ ID NO: 7 - DNA, 46 bp, synthetic construct
  source 1..46: mol_type = other DNA
agaaggagatataactatgcgagttctattgattgcctttttattg

SEQ ID NO: 8 - DNA, 45 bp, synthetic construct
  source 1..45: mol_type = other DNA
agaaggagatataactatgcagaaagattttttaaatgaaacaac